European Patent Specification EP 3 277 676 B1, published March 22, 2023. Title: SUBSTITUTED QUINAZOLINE DERIVATIVES AS DNA METHYLTRANSFERASE INHIBITORS. Applicant: PIERRE FABRE MEDICAMENT CENTRE NATIONAL DE LA RECHERCHE SCIENTIFIQUE (CNRS) SAPIENZA UNIVERSITA DI ROMA. The sequence listing filed with the application follows.

SEQUENCE LISTING (2 sequences)

SEQ ID NO: 1 - DNA, 33 bp, Artificial Sequence
  DNA duplex
  modified_base (4)..(4): methylCys
  modified_base (7)..(7): methylCys
  modified_base (12)..(12): methylCys
  modified_base (14)..(14): methylCys
  modified_base (19)..(19): methylCys
  modified_base (21)..(21): methylCys
  modified_base (25)..(25): methylCys
  modified_base (30)..(30): methylCys
gatcgccgatgcgcgaatcgcgatcgatgcgat

SEQ ID NO: 2 - DNA, 33 bp, Artificial Sequence
  DNA duplex
  misc_binding (1)..(1): Biotinylation
atcgcatcgatcgcgattcgcgcatcggcgatc